European Patent Application EP 4 775 678 A1, published July 15, 2026. Title: 애기장대 유래의 쓰레오닌 탈수효소가 도입된 미생물 및 이를 이용한 분지쇄 아미노산 생산 방법. Applicant: 씨제이제일제당 주식회사. The sequence listing filed with the application follows.

SEQUENCE LISTING (51 sequences)

SEQ ID NO: 1 - DNA, 38 bp, synthetic construct
  source 1..38: mol_type = other DNA
gctcggtacccggggatccggtgattgcgagcaatccc

SEQ ID NO: 2 - DNA, 35 bp, synthetic construct
  source 1..35: mol_type = other DNA
tatgtggttgactagtgtaatcctctcctagaatt

SEQ ID NO: 3 - DNA, 35 bp, synthetic construct
  source 1..35: mol_type = other DNA
cactagtcaaccacatagctgaaggccacctcaat

SEQ ID NO: 4 - DNA, 42 bp, synthetic construct
  source 1..42: mol_type = other DNA
gcctgcaggtcgactctagatgaacacaccggaaactactcc

SEQ ID NO: 5 - DNA, 24 bp, synthetic construct
  source 1..24: mol_type = other DNA
gcattgttctacaaagagctcgtt

SEQ ID NO: 6 - DNA, 20 bp, synthetic construct
  source 1..20: mol_type = other DNA
gagaactggctatcgatggc

SEQ ID NO: 7 - DNA, 38 bp, synthetic construct; identical to SEQ ID NO: 1
  source 1..38: mol_type = other DNA

SEQ ID NO: 8 - DNA, 30 bp, synthetic construct
  source 1..30: mol_type = other DNA
ggttgactagtgtaatcctctcctagaatt

SEQ ID NO: 9 - DNA, 32 bp, synthetic construct
  source 1..32: mol_type = other DNA
acatagctgaaggccacctcaatcgaggtggc

SEQ ID NO: 10 - DNA, 42 bp, synthetic construct; identical to SEQ ID NO: 4
  source 1..42: mol_type = other DNA

SEQ ID NO: 11 - DNA, 38 bp, synthetic construct
  source 1..38: mol_type = other DNA
ggattacactagtcaaccatgtccatgaccccgcctcc

SEQ ID NO: 12 - DNA, 39 bp, synthetic construct
  source 1..39: mol_type = other DNA
aggtggccttcagctatgtttagtgcatgagtagtttaa

SEQ ID NO: 13 - protein, 592 aa, Arabidopsis thaliana
  source 1..592: note = ilvA
MNSVQLPTAQSSLRSHIHRPSKPVVGFTHFSSRSRIAVAVLSRDETSMTPPPPKLPLPRLKVSPNSLQYPAGYLGAVPERTNEAENGSIAEAMEYLTNILSTKVYDIAIESPLQLAKKLSKRLGVRMYLKREDLQPVFSFKLRGAYNMMVKLPADQLAKGVICSSAGNHAQGVALSASKLGCTAVIVMPVTTPEIKWQAVENLGATVVLFGDSYDQAQAHAKIRAEEEGLTFIPPFDHPDVIAGQGTVGMEITRQAKGPLHAIFVPVGGGGLIAGIAAYVKRVSPEVKIIGVEPADANAMALSLHHGERVILDQVGGFADGVAVKEVGEETFRISRNLMDGVVLVTRDAICASIKDMFEEKRNILEPAGALALAGAEAYCKYYGLKDVNVVAITSGANMNFDKLRIVTELANVGRQQEAVLATLMPEKPGSFKQFCELVGPMNISEFKYRCSSEKEAVVLYSVGVHTAGELKALQKRMESSQLKTVNLTTSDLVKDHLRYLMGGRSTVGDEVLCRFTFPERPGALMNFLDSFSPRWNITLFHYRGQGETGANVLVGIQVPEQEMEEFKNRAKALGYDYFLVSDDDYFKLLMH

SEQ ID NO: 14 - DNA, 1779 bp, Arabidopsis thaliana
  source 1..1779: mol_type = genomic DNA; note = ilvA
atgaatagcgtccagcttcccacggcccaaagctcgcttaggtcccacatccaccgcccatccaaaccagtcgtgggattcacccatttctcctcacgctcccggattgctgtagcggtgctgtctcgggatgagacctccatgaccccgcctccgccgaaactcccgctccctcgtctaaaggtgtctccaaactcattgcagtacccagctggttatctcggtgctgttcccgaacgcaccaacgaagctgaaaacggctctatcgctgaagccatggaataccttactaacatcttgtctaccaaggtttatgacattgccatcgagagtcccctccaacttgcaaagaagctgtcgaaaaggttgggagtccgaatgtaccttaaacgtgaggatttgcaaccagtttttagcttcaaactgcgtggagcttacaacatgatggtcaaattgccagcagaccaattggcgaagggtgttatctgctcctctgcgggaaaccacgcccagggtgttgcattaagcgccagtaagttgggctgcacggctgtcattgtcatgcccgtgacaacaccagagatcaagtggcaggcagttgaaaacctgggcgccacggtggtgcttttcggcgattcctacgatcaagcacaggcgcatgcgaaaatccgcgcggaggaagagggactcaccttcatccctccgtttgatcacccagatgtgatcgccggccaaggaactgtcggcatggaaatcactcgacaagccaagggtccactgcatgcgattttcgtcccagtgggaggcggagggctgattgcaggcatcgctgcatatgtcaagcgcgtttctccggaagtaaagatcattggcgtggagcctgcggacgcaaatgcgatggctttgtcgctgcaccacggtgagagagtgattctcgatcaggttggtggttttgctgacggtgtagccgtgaaggaagtgggtgaagaaaccttccgcatttcccgcaaccttatggatggggtagtgctcgtgactcgcgacgcaatttgtgcaagcatcaaggacatgttcgaggagaagcgtaatattctcgaacctgcgggtgctctggcactagctggggctgaggcctactgcaaatattacggcctgaaagacgtcaacgtggttgctatcacgtctggcgccaacatgaattttgacaagctgcgcatcgtcaccgaattagccaatgtgggccgtcagcaagaagcagtcttggcgacactgatgccagaaaagcctggctcctttaagcagttctgtgaacttgttggccccatgaacatctccgaattcaagtaccgctgttcatccgaaaaagaggcggttgtactgtattcggtgggagtgcacaccgcaggcgagttgaaggctttgcagaagcgcatggagtcgtcacagctcaagaccgtcaatctcaccacctccgatctcgtaaaagatcatttgcgctatctgatgggcggccggagcaccgttggcgacgaggttctctgccgttttactttccccgagcgtcctggtgcgttgatgaattttcttgattcctttagtccccgctggaacatcaccctgttccactaccgagggcagggggaaacaggtgcaaacgttctggtcggcattcaggtgcctgagcaggaaatggaagagttcaaaaaccgcgcaaaagcccttggctacgactacttcctggtttctgatgacgattactttaaactactcatgcactaa

SEQ ID NO: 15 - protein, 547 aa, Arabidopsis thaliana
  source 1..547: note = ilvA w/o Transit peptide
MSMTPPPPKLPLPRLKVSPNSLQYPAGYLGAVPERTNEAENGSIAEAMEYLTNILSTKVYDIAIESPLQLAKKLSKRLGVRMYLKREDLQPVFSFKLRGAYNMMVKLPADQLAKGVICSSAGNHAQGVALSASKLGCTAVIVMPVTTPEIKWQAVENLGATVVLFGDSYDQAQAHAKIRAEEEGLTFIPPFDHPDVIAGQGTVGMEITRQAKGPLHAIFVPVGGGGLIAGIAAYVKRVSPEVKIIGVEPADANAMALSLHHGERVILDQVGGFADGVAVKEVGEETFRISRNLMDGVVLVTRDAICASIKDMFEEKRNILEPAGALALAGAEAYCKYYGLKDVNVVAITSGANMNFDKLRIVTELANVGRQQEAVLATLMPEKPGSFKQFCELVGPMNISEFKYRCSSEKEAVVLYSVGVHTAGELKALQKRMESSQLKTVNLTTSDLVKDHLRYLMGGRSTVGDEVLCRFTFPERPGALMNFLDSFSPRWNITLFHYRGQGETGANVLVGIQVPEQEMEEFKNRAKALGYDYFLVSDDDYFKLLMH

SEQ ID NO: 16 - DNA, 1644 bp, Arabidopsis thaliana
  source 1..1644: mol_type = genomic DNA; note = ilvA w/o Transit peptide
atgtccatgaccccgcctccgccgaaactcccgctccctcgtctaaaggtgtctccaaactcattgcagtacccagctggttatctcggtgctgttcccgaacgcaccaacgaagctgaaaacggctctatcgctgaagccatggaataccttactaacatcttgtctaccaaggtttatgacattgccatcgagagtcccctccaacttgcaaagaagctgtcgaaaaggttgggagtccgaatgtaccttaaacgtgaggatttgcaaccagtttttagcttcaaactgcgtggagcttacaacatgatggtcaaattgccagcagaccaattggcgaagggtgttatctgctcctctgcgggaaaccacgcccagggtgttgcattaagcgccagtaagttgggctgcacggctgtcattgtcatgcccgtgacaacaccagagatcaagtggcaggcagttgaaaacctgggcgccacggtggtgcttttcggcgattcctacgatcaagcacaggcgcatgcgaaaatccgcgcggaggaagagggactcaccttcatccctccgtttgatcacccagatgtgatcgccggccaaggaactgtcggcatggaaatcactcgacaagccaagggtccactgcatgcgattttcgtcccagtgggaggcggagggctgattgcaggcatcgctgcatatgtcaagcgcgtttctccggaagtaaagatcattggcgtggagcctgcggacgcaaatgcgatggctttgtcgctgcaccacggtgagagagtgattctcgatcaggttggtggttttgctgacggtgtagccgtgaaggaagtgggtgaagaaaccttccgcatttcccgcaaccttatggatggggtagtgctcgtgactcgcgacgcaatttgtgcaagcatcaaggacatgttcgaggagaagcgtaatattctcgaacctgcgggtgctctggcactagctggggctgaggcctactgcaaatattacggcctgaaagacgtcaacgtggttgctatcacgtctggcgccaacatgaattttgacaagctgcgcatcgtcaccgaattagccaatgtgggccgtcagcaagaagcagtcttggcgacactgatgccagaaaagcctggctcctttaagcagttctgtgaacttgttggccccatgaacatctccgaattcaagtaccgctgttcatccgaaaaagaggcggttgtactgtattcggtgggagtgcacaccgcaggcgagttgaaggctttgcagaagcgcatggagtcgtcacagctcaagaccgtcaatctcaccacctccgatctcgtaaaagatcatttgcgctatctgatgggcggccggagcaccgttggcgacgaggttctctgccgttttactttccccgagcgtcctggtgcgttgatgaattttcttgattcctttagtccccgctggaacatcaccctgttccactaccgagggcagggggaaacaggtgcaaacgttctggtcggcattcaggtgcctgagcaggaaatggaagagttcaaaaaccgcgcaaaagcccttggctacgactacttcctggtttctgatgacgattactttaaactactcatgcactaa

SEQ ID NO: 17 - DNA, 34 bp, synthetic construct
  source 1..34: mol_type = other DNA
ttacactagtcaaccatggctgactcgcaacccc

SEQ ID NO: 18 - DNA, 43 bp, synthetic construct
  source 1..43: mol_type = other DNA
ggtggccttcagctatgtctaacccgccaaaaagaacctgaac

SEQ ID NO: 19 - protein, 514 aa, Escherichia coli [sequence omitted]

SEQ ID NO: 20 - DNA, 1545 bp, Escherichia coli
  source 1..1545: mol_type = genomic DNA; note = ilvA
atggctgactcgcaacccctgtccggtgctccggaaggtgccgaatatttaagagcagtgctgcgcgcgccggtttacgaggcggcgcaggttacgccgctacaaaaaatggaaaaactgtcgtcgcgtcttgataacgtcattctggtgaagcgcgaagatcgccagccagtgcacagctttaagctgcgcggcgcatacgccatgatggcgggcctgacggaagaacagaaagcgcacggcgtgatcactgcttctgcgggtaaccacgcgcagggcgtcgcgttttcttctgcgcggttaggcgtgaaggccctgatcgttatgccaaccgccaccgccgacatcaaagtcgacgcggtgcgcggcttcggcggcgaagtgctgctccacggcgcgaactttgatgaagcgaaagccaaagcgatcgaactgtcacagcagcaggggttcacctgggtgccgccgttcgaccatccgatggtgattgccgggcaaggcacgctggcgctggaactgctccagcaggacgcccatctcgaccgcgtatttgtgccagtcggcggcggcggtctggctgctggcgtggcggtgctgatcaaacaactgatgccgcaaatcaaagtgatcgccgtagaagcggaagactccgcctgcctgaaagcagcgctggatgcgggtcatccggttgatctgccgcgcgtagggctatttgctgaaggcgtagcggtaaaacgcatcggtgacgaaaccttccgtttatgccaggagtatctcgacgacatcatcaccgtcgatagcgatgcgatctgtgcggcgatgaaggatttattcgaagatgtgcgcgcggtggcggaaccctctggcgcgctggcgctggcgggaatgaaaaaatatatcgccctgcacaacattcgcggcgaacggctggcgcatattctttccggtgccaacgtgaacttccacggcctgcgctacgtctcagaacgctgcgaactgggcgaacagcgtgaagcgttgttggcggtgaccattccggaagaaaaaggcagcttcctcaaattctgccaactgcttggcgggcgttcggtcaccgagttcaactaccgttttgccgatgccaaaaacgcctgcatctttgtcggtgtgcgcctgagccgcggcctcgaagagcgcaaagaaattttgcagatgctcaacgacggcggctacagcgtggttgatctctccgacgacgaaatggcgaagctacacgtgcgctatatggtcggcggacgtccatcgcatccgttgcaggaacgcctctacagcttcgaattcccggaatcaccgggcgcgctgctgcgcttcctcaacacgctgggtacgtactggaacatttctttgttccactatcgcagccatggcaccgactacgggcgcgtactggcggcgttcgaacttggcgaccatgaaccggatttcgaaacccggctgaatgagctgggctacgattgccacgacgaaaccaataacccggcgttcaggttctttttggcgggttag

SEQ ID NO: 21 - DNA, 38 bp, synthetic construct
  source 1..38: mol_type = other DNA
gattacactagtcaaccatgctgtcctccccagcaacc

SEQ ID NO: 22 - DNA, 40 bp, synthetic construct
  source 1..40: mol_type = other DNA
gtggccttcagctatgttcagtgcatgatcagctggtatg

SEQ ID NO: 23 - protein, 606 aa, Solanum lycopersicum
  source 1..606: note = ilvA
MEVLRFTAVKSLNSCVRPEFTAMSSVIVPISTVKVSGTRKSKKKALICAKATEILSSPATVTEPLKAEPAEAPVPLLRVSPSSLQCEPGYLLPNSPVLGTGGVTGYEYLTNILSSKVYDVAYETPLQKAPKLSERLGVNVWLKREDLQPVFSFKIRGAYNMMAKLPKEQLEKGVICSSAGNHAQGVALSAQRLGCDAVIVMPVTTPDIKWKSVKRLGATVVLVGDSYDEAQAYAKKRAESEGRTFIPPFDHPDVIVGQGTVGMEINRQLKDNIHAIFVPVGGGGLIAGIAAYLKRVAPDIKIIGVEPLDANALALSLHHGQRVMLDQVGGFADGVAVKVVGEETYRLCEELIDGVVLVGRDAICASIKDMFEEKRSILEPAGALALAGAEAYCKYYGLKGENVVAITSGANMNFDRLRLVTELADVGRQREAVLATFMPEDPGSFKKFAEMVGPMNITEFKYRYNSDKERALVLYSVGLHTILELEGMVERMESADLQTINLTDNDLVKDHLRHLMGGRTNVHNELLCRFTFPEKPGALMKFLDAFSPRWNISLFHYRAQGDTGANVLVGIQVPPDEVVEFEGRADSLGYEYAMESLNEAYQLIMH

SEQ ID NO: 24 - DNA, 1821 bp, Solanum lycopersicum
  source 1..1821: mol_type = genomic DNA; note = ilvA
atggaagtgctgcgcttcaccgcagtgaagtccctgaactcctgcgtccgtccagaattcaccgcaatgtcctccgtgatcgtcccaatttccaccgtcaaggtctccggtacccgcaagtccaagaagaaggcattgatctgcgcaaaggcaaccgagatcctgtcctccccagcaaccgtgaccgaaccattgaaggcagaaccagctgaagcaccagtgccactgctgcgcgtcagcccatcctccctgcagtgcgaaccaggttacctgctgccaaactccccagttctgggcaccggcggcgtcaccggctacgagtacctgaccaacatcctgtcctccaaggtctacgatgttgcatacgaaacccctctgcagaaggctcctaagctcagcgaacgcctgggcgtgaacgtctggctgaagcgcgaggatctccagccagttttctccttcaagatccgcggcgcatacaacatgatggcgaagctgcctaaggaacagctcgaaaagggcgtgatctgctcctccgcaggtaaccacgcacagggcgtggcactgtccgcacagcgcttgggttgcgatgctgtgatcgtcatgccagtcaccacccctgatatcaagtggaagtccgtgaagcgcctcggtgcaaccgtggtcctcgtgggcgatagctacgatgaagcccaggcatacgcaaagaagcgtgctgaatccgaaggtcgcaccttcatccctcctttcgatcaccctgatgtcatcgtgggtcagggcaccgtgggcatggagatcaaccgccagctgaaggacaacatccacgcgattttcgttccagtcggcggcggcggcctgattgctggcatcgctgcatacctgaagcgcgtcgcaccagatatcaagatcatcggcgtcgaaccactggatgctaacgcactggcactgtccctgcaccacggccagcgcgtcatgctggatcaggtcggcggcttcgcagatggcgtggctgtgaaggtcgtgggcgaagaaacctaccgcctctgcgaagaactcatcgatggtgtggtcctcgttggccgcgatgcaatctgcgcttctattaaggacatgttcgaagagaagcgcagcatcctggaacctgcaggcgcactggctctggcaggcgctgaggcctactgcaaatactacggcctcaagggcgaaaacgtggtggcaatcacctccggcgcaaacatgaacttcgatcgcctccgcctggtcaccgaactggcagatgtgggccgccagcgcgaagcagtgctggctaccttcatgccagaggacccaggctccttcaagaagttcgctgaaatggtcggcccaatgaacatcaccgagttcaagtaccgttacaactccgataaggaacgcgctctggtcctgtactccgtcggcctgcacaccatccttgagcttgaaggcatggtggaacgcatggaatccgccgatctgcagaccatcaacctgaccgacaacgatctcgtgaaggaccacctgcgccacctgatgggcggtcgtaccaacgttcacaacgaactgctgtgccgcttcaccttcccagaaaagccaggcgcactcatgaagttccttgatgcattctccccacgttggaacatctccctgttccactaccgcgcacagggcgataccggcgcaaacgtgttggtgggcatccaggtgccaccagatgaagtcgttgaattcgaaggccgcgcagattccctgggctacgaatacgcaatggaatctctgaacgaagcataccagctgatcatgcactga

SEQ ID NO: 25 - protein, 553 aa, Solanum lycopersicum
  source 1..553: note = ilvA w/o Transit peptide
MLSSPATVTEPLKAEPAEAPVPLLRVSPSSLQCEPGYLLPNSPVLGTGGVTGYEYLTNILSSKVYDVAYETPLQKAPKLSERLGVNVWLKREDLQPVFSFKIRGAYNMMAKLPKEQLEKGVICSSAGNHAQGVALSAQRLGCDAVIVMPVTTPDIKWKSVKRLGATVVLVGDSYDEAQAYAKKRAESEGRTFIPPFDHPDVIVGQGTVGMEINRQLKDNIHAIFVPVGGGGLIAGIAAYLKRVAPDIKIIGVEPLDANALALSLHHGQRVMLDQVGGFADGVAVKVVGEETYRLCEELIDGVVLVGRDAICASIKDMFEEKRSILEPAGALALAGAEAYCKYYGLKGENVVAITSGANMNFDRLRLVTELADVGRQREAVLATFMPEDPGSFKKFAEMVGPMNITEFKYRYNSDKERALVLYSVGLHTILELEGMVERMESADLQTINLTDNDLVKDHLRHLMGGRTNVHNELLCRFTFPEKPGALMKFLDAFSPRWNISLFHYRAQGDTGANVLVGIQVPPDEVVEFEGRADSLGYEYAMESLNEAYQLIMH

SEQ ID NO: 26 - DNA, 1662 bp, Solanum lycopersicum
  source 1..1662: mol_type = genomic DNA; note = ilvA w/o Transit peptide
atgctgtcctccccagcaaccgtgaccgaaccattgaaggcagaaccagctgaagcaccagtgccactgctgcgcgtcagcccatcctccctgcagtgcgaaccaggttacctgctgccaaactccccagttctgggcaccggcggcgtcaccggctacgagtacctgaccaacatcctgtcctccaaggtctacgatgttgcatacgaaacccctctgcagaaggctcctaagctcagcgaacgcctgggcgtgaacgtctggctgaagcgcgaggatctccagccagttttctccttcaagatccgcggcgcatacaacatgatggcgaagctgcctaaggaacagctcgaaaagggcgtgatctgctcctccgcaggtaaccacgcacagggcgtggcactgtccgcacagcgcttgggttgcgatgctgtgatcgtcatgccagtcaccacccctgatatcaagtggaagtccgtgaagcgcctcggtgcaaccgtggtcctcgtgggcgatagctacgatgaagcccaggcatacgcaaagaagcgtgctgaatccgaaggtcgcaccttcatccctcctttcgatcaccctgatgtcatcgtgggtcagggcaccgtgggcatggagatcaaccgccagctgaaggacaacatccacgcgattttcgttccagtcggcggcggcggcctgattgctggcatcgctgcatacctgaagcgcgtcgcaccagatatcaagatcatcggcgtcgaaccactggatgctaacgcactggcactgtccctgcaccacggccagcgcgtcatgctggatcaggtcggcggcttcgcagatggcgtggctgtgaaggtcgtgggcgaagaaacctaccgcctctgcgaagaactcatcgatggtgtggtcctcgttggccgcgatgcaatctgcgcttctattaaggacatgttcgaagagaagcgcagcatcctggaacctgcaggcgcactggctctggcaggcgctgaggcctactgcaaatactacggcctcaagggcgaaaacgtggtggcaatcacctccggcgcaaacatgaacttcgatcgcctccgcctggtcaccgaactggcagatgtgggccgccagcgcgaagcagtgctggctaccttcatgccagaggacccaggctccttcaagaagttcgctgaaatggtcggcccaatgaacatcaccgagttcaagtaccgttacaactccgataaggaacgcgctctggtcctgtactccgtcggcctgcacaccatccttgagcttgaaggcatggtggaacgcatggaatccgccgatctgcagaccatcaacctgaccgacaacgatctcgtgaaggaccacctgcgccacctgatgggcggtcgtaccaacgttcacaacgaactgctgtgccgcttcaccttcccagaaaagccaggcgcactcatgaagttccttgatgcattctccccacgttggaacatctccctgttccactaccgcgcacagggcgataccggcgcaaacgtgttggtgggcatccaggtgccaccagatgaagtcgttgaattcgaaggccgcgcagattccctgggctacgaatacgcaatggaatctctgaacgaagcataccagctgatcatgcactga

SEQ ID NO: 27 - DNA, 37 bp, synthetic construct
  source 1..37: mol_type = other DNA
attacactagtcaaccatgttctccccagaagagacc

SEQ ID NO: 28 - DNA, 40 bp, synthetic construct
  source 1..40: mol_type = other DNA
ggtggccttcagctatgttcagtgcatcaggacttcgtag

SEQ ID NO: 29 - protein, 613 aa, Spinacia oleracea
  source 1..613: note = ilvA
MSLSFLHSTGGGAATTTTTYDYLSSHHRPNIHPNSSLLHLPKLYRRHALVVKATVFSPEETLVKKPPPSSSPTPAPLRVVSTDSLVYESGFLGAVPEYSSPESSDDGSAAAMECLTNILSSKVYDIAVQSPLQLAEKLSERLGNNVWLKREDLQPVFSFKLRGAYNMMVKLPKEQLERGVICSSAGNHAQGVALSAKKLGCDAVIVMPVTTPEIKWKSVKRLGATVVLVGDSYDEAQAYAKNRAEEEGRTFIPPFDHPDVIMGQGTVGMEIVNQAKGRPLHAIFVPVGGGGLIAGIAAYVKRIQPEVKIIGVEPADANAMALSLHHGQRIMLDKVGGFADGVAVKVVGEETFRICKELIDGVVLVNRDAICASIKNMFEEKRSILEPAGALALAGAEAYCKYYGIKNENVVAITSGANMNFDRLRLVTELADVGRQREAVLATFMPEDPGSFKKFAEMVGPMNITEFKYRYNSAKEEALVLYSVGHHTVSELEALKERMESSKLRTINLTNNDLVKDHLRHLMGGRSDVQNELLCRFVFPERPGALMKFLDVFSPRWNISLFHYRAQGEAGANVLVGIQVPSSEMDEFRERADNLGFMYAIESDNEVYEVLMH

SEQ ID NO: 30 - DNA, 1842 bp, Spinacia oleracea
  source 1..1842: mol_type = genomic DNA; note = ilvA
atgtccctgtccttcctccactccaccggcggcggtgctgcaaccaccaccaccacctacgattacctctcctcccaccaccgcccaaacatccacccaaactcctccctgcttcacctgccaaagctgtaccgccgccacgctctggtggtgaaggcaaccgtgttctccccagaagagaccctggttaagaagccaccaccatcctcctccccaacccctgcaccactgcgcgtggtctccaccgattccctggtgtacgagtccggcttcctgggtgcagttccagaatactcctccccagaatcctccgatgacggttccgcagctgcaatggaatgcctgaccaacatcctgtcctccaaggtgtacgatatcgcagtgcagtccccacttcagctggccgaaaagctgtccgagcgtctgggcaacaacgtgtggctgaagcgcgaggatctgcagccggttttctccttcaagctgcgcggcgcatacaacatgatggtgaagctgccaaaggaacaacttgagcgcggcgtgatctgctcctctgcaggtaaccacgcacagggtgttgctctgtccgcaaagaagcttggctgcgatgctgttatcgtgatgccggtgaccaccccagaaatcaagtggaagtccgtgaagcgcctgggcgctaccgtcgtccttgttggcgattcctacgatgaggcacaggcatacgcaaagaaccgcgcagaagaagagggccgcactttcatcccaccgttcgatcacccagatgtgatcatgggtcagggtaccgtgggcatggaaatcgtgaaccaggcaaagggccgcccactgcacgcaatcttcgtcccagttggcggcggtggcctgatcgctggcatcgcagcctacgtgaagcgtatccagccagaagttaagatcatcggcgtggagccagctgatgcaaacgcaatggcactgtccctgcaccacggccagcgcatcatgctggataaggtgggcggcttcgcagatggcgtcgcagtcaaggtggtgggcgaagaaaccttccgcatctgcaaggagctgatcgatggcgtcgtcctcgtgaaccgcgatgcaatctgcgcttccatcaaaaacatgttcgaagaaaagcgctccatcctggagccagcaggcgcactcgctctggcaggcgcagaagcatactgcaagtactacggcatcaagaacgagaacgtggtcgctatcacctccggcgctaacatgaacttcgatcgcctgcgcctggtcaccgaacttgctgatgtcggtcgccagcgcgaggctgtgctggcaaccttcatgccggaggacccaggctccttcaagaagttcgctgaaatggtcggtccaatgaacatcaccgaattcaagtaccgctacaactccgcaaaggaagaggcactggtcctgtactccgtgggccaccacaccgtgtccgagctggaagcacttaaggagcgcatggaatcctccaagctgcgcaccatcaacctgaccaacaacgacctggtgaaggatcacctccgtcacctgatgggcggccgttctgatgtgcagaacgagcttctgtgccgcttcgtgttcccagagcgcccaggcgcactgatgaagttcctcgatgtgttctccccacgctggaacatctccctgttccactaccgcgctcagggcgaagcaggcgcaaacgtcctggtgggtatccaggtgccatcctccgaaatggatgaattccgcgaacgcgcagataacctgggcttcatgtacgcaatcgaatccgataacgaagtctacgaagtcctgatgcactga

SEQ ID NO: 31 - protein, 559 aa, Spinacia oleracea
  source 1..559: note = ilvA w/o Transit peptide
MFSPEETLVKKPPPSSSPTPAPLRVVSTDSLVYESGFLGAVPEYSSPESSDDGSAAAMECLTNILSSKVYDIAVQSPLQLAEKLSERLGNNVWLKREDLQPVFSFKLRGAYNMMVKLPKEQLERGVICSSAGNHAQGVALSAKKLGCDAVIVMPVTTPEIKWKSVKRLGATVVLVGDSYDEAQAYAKNRAEEEGRTFIPPFDHPDVIMGQGTVGMEIVNQAKGRPLHAIFVPVGGGGLIAGIAAYVKRIQPEVKIIGVEPADANAMALSLHHGQRIMLDKVGGFADGVAVKVVGEETFRICKELIDGVVLVNRDAICASIKNMFEEKRSILEPAGALALAGAEAYCKYYGIKNENVVAITSGANMNFDRLRLVTELADVGRQREAVLATFMPEDPGSFKKFAEMVGPMNITEFKYRYNSAKEEALVLYSVGHHTVSELEALKERMESSKLRTINLTNNDLVKDHLRHLMGGRSDVQNELLCRFVFPERPGALMKFLDVFSPRWNISLFHYRAQGEAGANVLVGIQVPSSEMDEFRERADNLGFMYAIESDNEVYEVLMH

SEQ ID NO: 32 - DNA, 1680 bp, Spinacia oleracea
  source 1..1680: mol_type = genomic DNA; note = ilvA w/o Transit peptide
atgttctccccagaagagaccctggttaagaagccaccaccatcctcctccccaacccctgcaccactgcgcgtggtctccaccgattccctggtgtacgagtccggcttcctgggtgcagttccagaatactcctccccagaatcctccgatgacggttccgcagctgcaatggaatgcctgaccaacatcctgtcctccaaggtgtacgatatcgcagtgcagtccccacttcagctggccgaaaagctgtccgagcgtctgggcaacaacgtgtggctgaagcgcgaggatctgcagccggttttctccttcaagctgcgcggcgcatacaacatgatggtgaagctgccaaaggaacaacttgagcgcggcgtgatctgctcctctgcaggtaaccacgcacagggtgttgctctgtccgcaaagaagcttggctgcgatgctgttatcgtgatgccggtgaccaccccagaaatcaagtggaagtccgtgaagcgcctgggcgctaccgtcgtccttgttggcgattcctacgatgaggcacaggcatacgcaaagaaccgcgcagaagaagagggccgcactttcatcccaccgttcgatcacccagatgtgatcatgggtcagggtaccgtgggcatggaaatcgtgaaccaggcaaagggccgcccactgcacgcaatcttcgtcccagttggcggcggtggcctgatcgctggcatcgcagcctacgtgaagcgtatccagccagaagttaagatcatcggcgtggagccagctgatgcaaacgcaatggcactgtccctgcaccacggccagcgcatcatgctggataaggtgggcggcttcgcagatggcgtcgcagtcaaggtggtgggcgaagaaaccttccgcatctgcaaggagctgatcgatggcgtcgtcctcgtgaaccgcgatgcaatctgcgcttccatcaaaaacatgttcgaagaaaagcgctccatcctggagccagcaggcgcactcgctctggcaggcgcagaagcatactgcaagtactacggcatcaagaacgagaacgtggtcgctatcacctccggcgctaacatgaacttcgatcgcctgcgcctggtcaccgaacttgctgatgtcggtcgccagcgcgaggctgtgctggcaaccttcatgccggaggacccaggctccttcaagaagttcgctgaaatggtcggtccaatgaacatcaccgaattcaagtaccgctacaactccgcaaaggaagaggcactggtcctgtactccgtgggccaccacaccgtgtccgagctggaagcacttaaggagcgcatggaatcctccaagctgcgcaccatcaacctgaccaacaacgacctggtgaaggatcacctccgtcacctgatgggcggccgttctgatgtgcagaacgagcttctgtgccgcttcgtgttcccagagcgcccaggcgcactgatgaagttcctcgatgtgttctccccacgctggaacatctccctgttccactaccgcgctcagggcgaagcaggcgcaaacgtcctggtgggtatccaggtgccatcctccgaaatggatgaattccgcgaacgcgcagataacctgggcttcatgtacgcaatcgaatccgataacgaagtctacgaagtcctgatgcactga

SEQ ID NO: 33 - DNA, 41 bp, synthetic construct
  source 1..41: mol_type = other DNA
gattacactagtcaaccatggaagtgttctccttcaagctg

SEQ ID NO: 34 - DNA, 38 bp, synthetic construct
  source 1..38: mol_type = other DNA
gtggccttcagctatgttcatgcctttgggttgcgcag

SEQ ID NO: 35 - protein, 463 aa, Brachypodium distachyon
  source 1..463: note = ilvA
MEVFSFKLRGAYNMMAKLSQEQLDRGVICSSAGNHAQGVALSARRLGCDAVIVMPVTTPEIKWRSVERLGATVVLKGDSYDEAQSYAKLRCEQESRTFIPPFDHPDIIAGQGTVGMEIVRQLQGPLHAIFVPVGGGGLIAGIAAYVKRVRPEVKIIGVEPSDANAMALSLSHGQRVMLEHVGGFADGVAVKVVGEETFRLCQELVDGIVLVSRDAICASIKDMFEENRNILEPAGALALAGAEAYCKYYGLKGETLVAISSGANMNFDRLRLVTELADVGRKREAVLATFLPEVQGSFKKFAELVGPMNITEFKYRYDSNGKEALVLYSVGIYTDLELRAMMERMESSKLKTVNLTSNDLAKDHLRYFIGGRSEVKDELVYRFIFPERPGTLMQFLDALSPRWNISLFHYRAQGETGANVLVGIQVPPEDLDEFRSRADNLGYEYMSEMNNEIYNLLLRNPKA

SEQ ID NO: 36 - DNA, 1392 bp, Brachypodium distachyon
  source 1..1392: mol_type = genomic DNA; note = ilvA
atggaagtgttctccttcaagctgcgcggcgcatacaacatgatggctaagctgtcccaggaacagctggatcgtggcgtgatctgctcctctgctggcaaccacgcacagggcgtggcactgtccgctcgccgcctgggctgcgatgctgtgatcgtcatgccagttaccaccccagaaatcaagtggcgctccgtggaacgcctgggcgcaaccgtcgtgctgaagggcgattcctacgatgaagctcagtcctacgcaaagctgcgctgcgaacaggagtcccgcaccttcattccaccattcgatcacccagatatcatcgcaggtcagggcaccgtgggcatggaaatcgtgcgccagctccagggcccactgcacgcaatcttcgttccggttggcggcggcggcctcatcgcaggcatcgccgcatacgtgaagcgcgtgcgcccagaagtgaagatcatcggcgtcgaaccatccgatgcaaacgctatggctctctccctgtcccacggtcagcgcgtcatgctggaacacgtcggtggcttcgctgatggcgtggctgttaaggtggtgggcgaagagaccttccgtctgtgccaggaactggtcgatggcatcgttctcgtgtctcgcgatgctatctgcgcatccatcaaggacatgttcgaagaaaaccgcaacatcctggaaccagcaggcgctctggcactggcaggcgctgaagcttactgcaagtactacggcctgaagggcgagaccctggtggcaatctcctctggcgctaacatgaacttcgaccgcctgcgcctggtgaccgaactggcagatgtgggccgtaagcgtgaagcagttctggctaccttcctgccagaagtccagggctccttcaagaagttcgctgaactcgttggcccaatgaacatcaccgaattcaagtaccgctacgattccaacggcaaggaagcactggtgctgtactccgtgggcatctacaccgatctggaactgcgcgcaatgatggaacgcatggaatcctccaagcttaagaccgtgaacctgacctccaacgatctggcaaaggatcacctgcgctacttcatcggcggccgctccgaagttaaggacgaactggtgtaccgcttcatcttcccagaacgcccaggcaccctgatgcagttcctggatgcactgtccccacgctggaacatctctctgttccactaccgcgcacagggcgagaccggcgctaacgtcctggtgggcatccaggtgccaccagaagatctcgatgaattccgctcccgcgctgataacctgggctacgaatacatgtccgaaatgaacaacgaaatctacaacctgctgctgcgcaacccaaaggcatga

SEQ ID NO: 37 - DNA, 41 bp, synthetic construct
  source 1..41: mol_type = other DNA
cggggatcccccgggaggacggtactcaaatactaaacttc

SEQ ID NO: 38 - DNA, 38 bp, synthetic construct
  source 1..38: mol_type = other DNA
tgccgagtgtttcggtctttacagacacgagggacacg

SEQ ID NO: 39 - DNA, 31 bp, synthetic construct
  source 1..31: mol_type = other DNA
tgtctgtaaagaccgaaacactcggcatcaa

SEQ ID NO: 40 - DNA, 41 bp, synthetic construct
  source 1..41: mol_type = other DNA
cggggatcccccggggacaactacattattattataccaca

SEQ ID NO: 41 - protein, 436 aa, Corynebacterium glutamicum
  source 1..436: note = ilvA
MSETYVSEKSPGVMASGAELIRAADIQTAQARISSVIAPTPLQYCPRLSEETGAEIYLKREDLQDVRSYKIRGALNSGAQLTQEQRDAGIVAASAGNHAQGVAYVCKSLGVQGRIYVPVQTPKQKRDRIMVHGGEFVSLVVTGNNFDEASAAAHEDAERTGATLIEPFDARNTVIGQGTVAAEILSQLTSMGKSADHVMVPVGGGGLLAGVVSYMADMAPRTAIVGIEPAGAASMQAALHNGGPITLETVDPFVDGAAVKRVGDLNYTIVEKNQGRVHMMSATEGAVCTEMLDLYQNEGIIAEPAGALSIAGLKEMSFAPGSVVVCIISGGNNDVLRYAEIAERSLVHRGLKHYFLVNFPQKPGQLRHFLEDILGPDDDITLFEYLKRNNRETGTALVGIHLSEASGLDSLLERMEESAIDSRRLEPGTPEYEYLT

SEQ ID NO: 42 - DNA, 1311 bp, Corynebacterium glutamicum
  source 1..1311: mol_type = genomic DNA; note = ilvA
atgagtgaaacatacgtgtctgagaaaagtccaggagtgatggctagcggagcggagctgattcgtgccgccgacattcaaacggcgcaggcacgaatttcctccgtcattgcaccaactccattgcagtattgccctcgtctttctgaggaaaccggagcggaaatctaccttaagcgtgaggatctgcaggatgttcgttcctacaagatccgcggtgcgctgaactctggagcgcagctcactcaggagcagcgcgatgcaggtatcgttgccgcatctgcaggtaaccatgcccagggcgtggcctatgtgtgcaagtccttgggcgttcagggacgcatctatgttcctgtgcagactccaaagcaaaagcgtgaccgcatcatggttcacggcggagagtttgtctccttggtggtcactggcaataacttcgacgaagcatcggctgcagcgcatgaagatgcagagcgcaccggcgcaacgctgatcgagcctttcgatgctcgcaacaccgtcatcggtcagggtacagtggctgctgagatcttgtcgcagctgacttccatgggcaagagtgcagatcacgtgatggttccagtcggcggtggcggacttcttgcaggtgtggtcagctacatggctgatatggcacctcgcactgcgatcgttggtatcgaaccagcgggagcagcatccatgcaggctgcattgcacaatggtggaccaatcactttggagactgttgatccctttgtggacggcgcagcagtcaaacgtgtcggagatctcaactacaccatcgtggagaagaaccagggtcgcgtgcacatgatgagcgcgaccgagggcgctgtgtgtactgagatgctcgatctttaccaaaacgaaggcatcatcgcggagcctgctggcgcgctgtctatcgctgggttgaaggaaatgtcctttgcacctggttctgtcgtggtgtgcatcatctctggtggcaacaacgatgtgctgcgttatgcggaaatcgctgagcgctccttggtgcaccgcggtttgaagcactacttcttggtgaacttcccgcaaaagcctggtcagttgcgtcacttcctggaagatatcctgggaccggatgatgacatcacgctgtttgagtacctcaagcgcaacaaccgtgagaccggtactgcgttggtgggtattcacttgagtgaagcatcaggattggattctttgctggaacgtatggaggaatcggcaattgattcccgtcgcctcgagccgggcacccctgagtacgaatacttgacctaa

SEQ ID NO: 43 - DNA, 1311 bp, Corynebacterium glutamicum
  source 1..1311: mol_type = genomic DNA; note = ilvA
atgagtgaaacatacgtgtctgagaaaagtccaggagtgatggctagcggagcggagctgattcgtgccgccgacattcaaacggcgcaggcacgaatttcctccgtcattgcaccaactccattgcagtattgccctcgtctttctgaggaaaccggagcggaaatctaccttaagcgtgaggatctgcaggatgttcgttcctacaagatccgcggtgcgctgaactctggagcgcagctcacccaagagcagcgcgatgcaggtatcgttgccgcatctgcaggtaaccatgcccagggcgtggcctatgtgtgcaagtccttgggcgttcagggacgcatctatgttcctgtgcagactccaaagcaaaagcgtgaccgcatcatggttcacggcggagagtttgtctccttggtggtcactggcaataacttcgacgaagcatcggctgcagcgcatgaagatgcagagcgcaccggcgcaacgctgatcgagcctttcgatgctcgcaacaccgtcatcggtcagggcaccgtggctgctgagatcttgtcgcagctgacttccatgggcaagagtgcagatcacgtgatggttccagtcggcggtggcggacttcttgcaggtgtggtcagctacatggctgatatggcacctcgcactgcgatcgttggtatcgaaccagcgggagcagcatccatgcaggctgcattgcacaatggtggaccaatcactttggagactgttgatccctttgtggacggcgcagcagtcaaacgtgtcggagatctcaactacaccatcgtggagaagaaccagggtcgcgtgcacatgatgagcgcgaccgagggcgctgtgtgtactgagatgctcgatctttaccaaaacgaaggcatcatcgcggagcctgctggcgcgctgtctatcgctgggttgaaggaaatgtcctttgcacctggttctgtcgtggtgtgcatcatctctggtggcaacaacgatgtgctgcgttatgcggaaatcgctgagcgctccttggtgcaccgcggtttgaagcactacttcttggtgaacttcccgcaaaagcctggtcagttgcgtcacttcctggaagatatcctgggaccggatgatgacatcacgctgtttgagtacctcaagcgcaacaaccgtgagaccggtactgcgttggtgggtattcacttgagtgaagcatcaggattggattctttgctggaacgtatggaggaatcggcaattgattcccgtcgcctcgagccgggcacccctgagtacgaatacttgacctaa

SEQ ID NO: 44 - DNA, 42 bp, synthetic construct
  source 1..42: mol_type = other DNA
tggccttcagctatgtcccgggcctactttggcataggtttt

SEQ ID NO: 45 - DNA, 41 bp, synthetic construct
  source 1..41: mol_type = other DNA
ggtcgactctagaggatcccctgtgtctcactccatcaacg

SEQ ID NO: 46 - DNA, 40 bp, synthetic construct
  source 1..40: mol_type = other DNA
gtgaattcgagctcggtacccatgatcgcggcgcctattc

SEQ ID NO: 47 - DNA, 42 bp, synthetic construct
  source 1..42: mol_type = other DNA
cctatgccaaagtaggcccgggacatagctgaaggccacctc

SEQ ID NO: 48 - DNA, 39 bp, synthetic construct
  source 1..39: mol_type = other DNA
cctatgccaaagtaggcccatgtccatgaccccgcctcc

SEQ ID NO: 49 - DNA, 42 bp, synthetic construct
  source 1..42: mol_type = other DNA
gaggtggccttcagctatgtcccttagtgcatgagtagttta

SEQ ID NO: 50 - DNA, 19 bp, synthetic construct
  source 1..19: mol_type = other DNA
ggtgattgcgagcaatccc

SEQ ID NO: 51 - DNA, 5802 bp, synthetic construct
  source 1..5802: mol_type = other DNA; note = pDC24 vector
gttcgcttgctgtccataaaaccgcccagtctagctatcgccatgtaagcccactgcaagctacctgctttctctttgcgcttgcgttttcccttgtccagatagcccagtagctgacattcatccggggtcagcaccgtttctgcggactggctttctacgtgttccgcttcctttagcagcccttgcgccctgagtgcttgcggcagcgtgaagctagcttttatcgccattcgccattcaggctgcgcaactgttgggaagggcgatcggtgcgggcctcttcgctattacgccagctggcgaaagggggatgtgctgcaaggcgattaagttgggtaacgccagggttttcccagtcacgacgttgtaaaacgacggccagtgaattcgagctcggtacccggggatcctctagagtcgacctgcaggcatgcaagcttggcgtaatcatggtcatagctgtttcctgtgtgaaattgttatccgctcacaattccacacaacatacgagccggaagcataaagtgtaaagcctggggtgcctaatgagtgagctaactcacattaattgcgttgcgctcactgcccgctttccagtcgggaaacctgtcgtgccagctgcattaatgaatcggccaacgcgcggggagaggcggtttgcgtattgggcgctcttccgcttcctcgctcactgactcgctgcgctcggtcgttcggctgcggcgagcggtatcagctcactcaaaggcggtaatacggttatccacagaatcaggggataacgcaggaaagaacatgtgagcaaaaggccagcaaaaggccaggaaccgtaaaaaggccgcgttgctggcgtttttccataggctccgcccccctgacgagcatcacaaaaatcgacgctcaagtcagaggtggcgaaacccgacaggactataaagataccaggcgtttccccctggaagctccctcgtgcgctctcctgttccgaccctgccgcttaccggatacctgtccgcctttctcccttcgggaagcgtggcgctttctcaatgctcacgctgtaggtatctcagttcggtgtaggtcgttcgctccaagctgggctgtgtgcacgaaccccccgttcagcccgaccgctgcgccttatccggtaactatcgtcttgagtccaacccggtaagacacgacttatcgccactggcagcagccactggtaacaggattagcagagcgaggtatgtaggcggtgctacagagttcttgaagtggtggcctaactacggctacactagaaggacagtatttggtatctgcgctctgctgaagccagttaccttcggaaaaagagttggtagctcttgatccggcaaacaaaccaccgctggtagcggtggtttttttgtttgcaagcagcagattacgcgcagaaaaaaaggatctcaagaagatcctttgatcttttctacggggtctgacgctcagtggaacgaaaactcacgttaagggattttggtcatgagattatcaaaaaggatcttcacctagatccttttggggtgggcgaagaactccagcatgagatccccgcgctggaggatcatccagccctgatagaaacagaagccactggagcacctcaaaaacaccatcatacactaaatcagtaagttggcagcatcacccgacgcactttgcgccgaataaatacctgtgacggaagatcacttcgcagaataaataaatcctggtgtccctgttgataccgggaagccctgggccaacttttggcgaaaatgagacgttgatcggcacgtaagaggttccaactttcaccataatgaaataagatcactaccgggcgtattttttgagttatcgagattttcaggagctgatagaaacagaagccactggagcacctcaaaaacaccatcatacactaaatcagtaagttggcagcatcacccgacgcactttgcgccgaataaatacctgtgacggaagatcacttcgcagaataaataaatcctggtgtccctgttgataccgggaagccctgggccaacttttggcgaaaatgagacgttgatcggcacgtaagaggttccaactttcaccataatgaaataagatcactaccgggcgtattttttgagttatcgagattttcaggagctctttggcatcgtctctcgcctgtcccctcagttcagtaatttcctgcatttgcctgtttccagtcggtagatattccacaaaacagcagggaagcagcgcttttccgctgcataaccctgcttcggggtcattatagcgattttttcggtatatccatcctttttcgcacgatatacaggattttgccaaagggttcgtgtagactttccttggtgtatccaacggcgtcagccgggcaggataggtgaagtaggcccacccgcgagcgggtgttccttcttcactgtcccttattcgcacctggcggtgctcaacgggaatcctgctctgcgaggctggccggctaccgccggcgtaacagatgagggcaagcggatggctgatgaaaccaagccaaccaggaagggcagcccacctatcaaggtgtactgccttccagacgaacgaagagcgattgaggaaaaggcggcggcggccggcatgagcctgtcggcctacctgctggccgtcggccagggctacaaaatcacgggcgtcgtggactatgagcacgtccgcgagggcgtcccggaaaacgattccgaagcccaacctttcatagaaggcggcggtggaatcgaaatctcgtgatggcaggttgggcgtcgcttggtcggtcatttcgaaaaaggttaggaatacggttagccatttgcctgcttttatatagttcatatgggattcacctttatgttgataagaaataaaagaaaatgccaataggatatcggcattttcttttgcgtttttatttgttaactgttaattgtccttgttcaaggatgctgtctttgacaacagatgttttcttgcctttgatgttcagcaggaagctcggcgcaaacgttgattgtttgtctgcgtagaatcctctgtttgtcatatagcttgtaatcacgacattgtttcctttcgcttgaggtacagcgaagtgtgagtaagtaaaggttacatcgttaggcggatcaagatccatttttaacacaaggccagttttgttcagcggcttgtatgggccagttaaagaattagaaacataaccaagcatgtaaatatcgttagacgtaatgccgtcaatcgtcatttttgatccgcgggagtcagtgaacaggtaccatttgccgttcattttaaagacgttcgcgcgttcaatttcatctgttactgtgttagatgcaatcagcggtttcatcacttttttcagtgtgtaatcatcgtttagctcaatcataccgagagcgccgtttgctaactcagccgtgcgttttttatcgctttgcagaagtttttgactttcttgacggaagaatgatgtgcttttgccatagtatgctttgttaaataaagattcttcgccttggtagccatcttcagttccagtgtttgcttcaaatactaagtatttgtggcctttatcttctacgtagtgaggatctctcagcgtatggttgtcgcctgagctgtagttgccttcatcgatgaactgctgtacattttgatacgtttttccgtcaccgtcaaagattgatttataatcctctacaccgttgatgttcaaagagctgtctgatgctgatacgttaacttgtgcagttgtcagtgtttgtttgccgtaatgtttaccggagaaatcagtgtagaataaacggatttttccgtcagatgtaaatgtggctgaacctgaccattcttgtgtttggtcttttaggatagaatcatttgcatcgaatttgtcgctgtctttaaagacgcggccagcgtttttccagctgtcaatagaagtttcgccgactttttgatagaacatgtaaatcgatgtgtcatccgcatttttaggatctccggctaatgcaaagacgatgtggtagccgtgatagtttgcgacagtgccgtcagcgttttgtaatggccagctgtcccaaacgtccaggccttttgcagaagagatatttttaattgtggacgaatcaaattcagaaacttgatatttttcatttttttgctgttcagggatttgcagcatatcatggcgtgtaatatgggaaatgccgtatgtttccttatatggcttttggttcgtttctttcgcaaacgcttgagttgcgcctcctgccagcagtgcggtagtaaaggttaatactgttgcttgttttgcaaactttttgatgttcatcgttcatgtctccttttttatgtactgtgttagcggtctgcttcttccagccctcctgtttgaagatggcaagttagttacgcacaataaaaaaagacctaaaatatgtaaggggtgacgccaaagtatacactttgccctttacacattttaggtcttgcctgctttatcagtaacaaacccgcgcgatttacttttcgacctcattctattagactctcgtttggattgcaactggtctattttcctcttttgtttgatagaaaatcataaaaggatttgcagactacgggcctaaagaactaaaaaatctatctgtttcttttcattctctgtattttttatagtttctgttgcatgggcataaagttgcctttttaatcacaattcagaaaatatcataatatctcatttcactaaataatagtgaacggcaggtatatgtgatgggttaaaaaggatcaccccagagtcccgctcagaagaactcgtcaagaaggcgatagaaggcgatgcgctgcgaatcgggagcggcgataccgtaaagcacgaggaagcggtcagcccattcgccgccaagctcttcagcaatatcacgggtagccaacgctatgtcctgatagcggtccgccacacccagccggccacagtcgatgaatccagaaaagcggccattttccaccatgatattcggcaagcaggcatcgccatgggtcacgacgagatcctcgccgtcgggcatccgcgccttgagcctggcgaacagttcggctggcgcgagcccctgatgctcttcgtccagatcatcctgatcgacaagaccggcttccatccgagtacgtgctcgctcgatgcgatgtttcgcttggtggtcgaatgggcaggtagccggatcaagcgtatgcagccgccgcattgcatcagccatgatggatactttctcggcaggagcaaggtgagatgacaggagatcctgccccggcacttcgcccaatagcagccagtcccttcccgcttcagtgacaacgtcgagacagctgcgcaaggaacgcccgtcgtggccagccacgatagccgcgctgcctcgtcttggagttcattcagggcaccggacaggtcggtcttgacaaaaagaaccgggcgcccctgcgctgacagccggaacacggcggcatcagagcagccgattgtctgttgtgcccagtcatagccgaatagcctctccacccaagcggccggagaacctgcgtgcaatccatcttgttcaatcatgcgaaacgatcctcatcctgtctcttgatcagatcttgatcccctgcgccatcagatccttggcggcaagaaagccatccagtttactttgcagggcttcccaaccttaccagagggcgccccagctggcaattccg